European Patent Application EP 4 428 237 A1, published September 11, 2024. Title: ISOLATED NUCLEIC ACID MOLECULE AND USE THEREOF. Applicant: Gritgen Therapeutics Limited. Application EP. The sequence listing filed with the application follows.

SEQUENCE LISTING (10 sequences)

SEQ ID NO: 1 - DNA, 266 bp, synthetic construct
  misc_feature 1..266: note = liver-specific expression regulatory element
  source 1..266: mol_type = other DNA
gctaaaatgggcaaacatgctgtttactgagctgggcacaatgacctttggcgagctggacagagggccgggtgctgacgtgcaggcgggtgggctgacctttaaacttgtttgctcctccgataaccggggtgaccttggttaatcattaaccagcaatggggttaataattttccagatctctctgagcaatagtataaaacaagaggtatcactcatttcagatcaggcttctcagaggtccccacccaatacatctccagtc

SEQ ID NO: 2 - DNA, 4425 bp, synthetic construct
  misc_feature 1..4425: note = Codon optimized polynucleotides encoding B-domain deleted FVIII
  source 1..4425: mol_type = other DNA
atgcagattgagctgagcacctgcttcttcctgtgcctgctgaggttctgcttctctgccaccaggagatactacctgggggctgtggagctgagctgggactacatgcagtctgacctgggggagctgcctgtggatgccaggttcccccccagagtgcccaagagcttccccttcaacacctctgtggtgtacaagaagaccctgtttgtggagttcactgaccacctgttcaacattgccaagcccaggcccccctggatgggcctgctgggccccaccatccaggctgaggtgtatgacactgtggtgatcaccctgaagaacatggccagccaccctgtgagcctgcatgctgtgggggtgagctactggaaggcctctgagggggctgagtatgatgaccagaccagccagagggagaaggaggatgacaaggtgttccctgggggcagccacacctatgtgtggcaggtgctgaaggagaatggccccatggcctctgaccccctgtgcctgacctacagctacctgagccatgtggacctggtgaaggacctgaactctggcctgattggggccctgctggtgtgcagggagggcagcctggccaaggagaagacccagaccctgcacaagttcatcctgctgtttgctgtgtttgatgagggcaagagctggcactctgaaaccaagaacagcctgatgcaggacagggatgctgcctctgccagggcctggcccaagatgcacactgtgaatggctatgtgaacaggagcctgcctggcctgattggctgccacaggaagtctgtgtactggcatgtgattggcatgggcaccacccctgaggtgcacagcatcttcctggagggccacaccttcctggtcaggaaccacaggcaggccagcctggagatcagccccatcaccttcctgactgcccagaccctgctgatggacctgggccagttcctgctgttctgccacatcagcagccaccagcatgatggcatggaggcctatgtgaaggtggacagctgccctgaggagccccagctgaggatgaagaacaatgaggaggctgaggactatgatgatgacctgactgactctgagatggatgtggtgaggtttgatgatgacaacagccccagcttcatccagatcaggtctgtggccaagaagcaccccaagacctgggtgcactacattgctgctgaggaggaggactgggactatgcccccctggtgctggcccctgatgacaggagctacaagagccagtacctgaacaatggcccccagaggattggcaggaagtacaagaaggtcaggttcatggcctacactgatgaaaccttcaagaccagggaggccatccagcatgagtctggcatcctgggccccctgctgtatggggaggtgggggacaccctgctgatcatcttcaagaaccaggccagcaggccctacaacatctacccacatggcatcactgatgtgaggcccctgtacagcaggaggctgcccaagggggtgaagcacctgaaggacttccccatcctgcctggggagatcttcaagtacaagtggactgtgactgtggaggatggccccaccaagtctgaccccaggtgcctgaccagatactacagcagctttgtgaacatggagagggacctggcctctggcctgattggccccctgctgatctgctacaaggagtctgtggaccagaggggcaaccagatcatgtctgacaagaggaatgtgatcctgttctctgtgtttgatgagaacaggagctggtacctgactgagaacatccagaggttcctgcccaaccctgctggggtgcagctggaggaccctgagttccaggccagcaacatcatgcacagcatcaatggctatgtgtttgacagcctgcagctgtctgtgtgcctgcatgaggtggcctactggtacatcctgagcattggggcccagactgacttcctgtctgtgttcttctctggctacaccttcaagcacaagatggtgtatgaggacaccctgaccctgttccccttctctggggagactgtgttcatgagcatggagaaccctggcctgtggattctgggctgccacaactctgacttcaggaacaggggcatgactgccctgctgaaagtctccagctgtgacaagaacactggggactactatgaggacagctatgaggacatctctgcctacctgctgagcaagaacaatgccattgagcccaggagcttcagccagaatgccactaatgtgtctaacaacagcaacaccagcaatgacagcaatgtgtctcccccagtgctgaagaggcaccagagggagatcaccaggaccaccctgcagtctgaccaggaggagattgactatgatgacaccatctctgtggagatgaagaaggaggactttgacatctacgacgaggacgagaaccagagccccaggagcttccagaagaagaccaggcactacttcattgctgctgtggagaggctgtgggactatggcatgagcagcagcccccatgtgctgaggaacagggcccagtctggctctgtgccccagttcaagaaggtggtgttccaggagttcactgatggcagcttcacccagcccctgtacagaggggagctgaatgagcacctgggcctgctgggcccctacatcagggctgaggtggaggacaacatcatggtgaccttcaggaaccaggccagcaggccctacagcttctacagcagcctgatcagctatgaggaggaccagaggcagggggctgagcccaggaagaactttgtgaagcccaatgaaaccaagacctacttctggaaggtgcagcaccacatggcccccaccaaggatgagtttgactgcaaggcctgggcctacttctctgatgtggacctggagaaggatgtgcactctggcctgattggccccctgctggtgtgccacaccaacaccctgaaccctgcccatggcaggcaggtgactgtgcaggagtttgccctgttcttcaccatctttgatgaaaccaagagctggtacttcactgagaacatggagaggaactgcagggccccctgcaacatccagatggaggaccccaccttcaaggagaactacaggttccatgccatcaatggctacatcatggacaccctgcctggcctggtgatggcccaggaccagaggatcaggtggtacctgctgagcatgggcagcaatgagaacatccacagcatccacttctctggccatgtgttcactgtgaggaagaaggaggagtacaagatggccctgtacaacctgtaccctggggtgtttgagactgtggagatgctgcccagcaaggctggcatctggagggtggagtgcctgattggggagcacctgcatgctggcatgagcaccctgttcctggtgtacagcaacaagtgccagacccccctgggcatggcctctggccacatcagggacttccagatcactgcctctggccagtatggccagtgggcccccaagctggccaggctgcactactctggcagcatcaatgcctggagcaccaaggagcccttcagctggatcaaggtggacctgctggcccccatgatcatccatggcatcaagacccagggggccaggcagaagttcagcagcctgtacatcagccagttcatcatcatgtacagcctggatggcaagaagtggcagacctacaggggcaacagcactggcacactgatggtgttctttggcaatgtggacagctctggcatcaagcacaacatcttcaacccccccatcattgccagatacatcaggctgcaccccacccactacagcatcaggagcaccctgaggatggagctgatgggctgtgacctgaacagctgcagcatgcccctgggcatggagagcaaggccatctctgatgcccagatcactgccagcagctacttcaccaacatgtttgccacctggagccccagcaaggccaggctgcacctgcagggcaggagcaatgcctggaggccccaggtcaacaaccccaaggagtggctgcaggtggacttccagaagaccatgaaggtgactggggtgaccacccagggggtgaagagcctgctgaccagcatgtatgtgaaggagttcctgatcagcagcagccaggatggccaccagtggaccctgttcttccagaatggcaaggtgaaggtgttccagggcaaccaggacagcttcacccctgtggtgaacagcctggacccccccctgctgaccagatacctgaggattcacccccagagctgggtgcaccagattgccctgaggatggaggtgctgggctgtgaggcccaggacctgtactga

SEQ ID NO: 3 - DNA, 96 bp, synthetic construct
  misc_feature 1..96: note = Ks13 polyA
  source 1..96: mol_type = other DNA
aatgcataaattgtaaatttattgacaaacaataaacaacaataaacaactgaaatgagtggctatgtattaaagaggggctggggggttgggttg

SEQ ID NO: 4 - DNA, 130 bp, synthetic construct
  misc_feature 1..130: note = 5'ITR (at the 5' end)
  source 1..130: mol_type = other DNA
ctgcgcgctcgctcgctcactgaggccgcccgggcaaagcccgggcgtcgggcgacctttggtcgcccggcctcagtgagcgagcgagcgcgcagagagggagtggccaactccatcactaggggttcct

SEQ ID NO: 5 - DNA, 130 bp, synthetic construct
  misc_feature 1..130: note = 3'ITR (at the 3' end)
  source 1..130: mol_type = other DNA
aggaacccctagtgatggagttggccactccctctctgcgcgctcgctcgctcactgaggccgggcgaccaaaggtcgcccgacgcccgggctttgcccgggcggcctcagtgagcgagcgagcgcgcag

SEQ ID NO: 6 - DNA, 4359 bp, synthetic construct
  misc_feature 1..4359: note = Wild-type nucleic acid molecule encoding B-domain deleted FVIII
  source 1..4359: mol_type = other DNA
atgcaaatagagctctccacctgcttctttctgtgccttttgcgattctgctttagtgccaccagaagatactacctgggtgcagtggaactgtcatgggactatatgcaaagtgatctcggtgagctgcctgtggacgcaagatttcctcctagagtgccaaaatcttttccattcaacacctcagtcgtgtacaaaaagactctgtttgtagaattcacggatcaccttttcaacatcgctaagccaaggccaccctggatgggtctgctaggtcctaccatccaggctgaggtttatgatacagtggtcattacacttaagaacatggcttcccatcctgtcagtcttcatgctgttggtgtatcctactggaaagcttctgagggagctgaatatgatgatcagaccagtcaaagggagaaagaagatgataaagtcttccctggtggaagccatacatatgtctggcaggtcctgaaagagaatggtccaatggcctctgacccactgtgccttacctactcatatctttctcatgtggacctggtaaaagacttgaattcaggcctcattggagccctactagtatgtagagaagggagtctggccaaggaaaagacacagaccttgcacaaatttatactactttttgctgtatttgatgaagggaaaagttggcactcagaaacaaagaactccttgatgcaggatagggatgctgcatctgctcgggcctggcctaaaatgcacacagtcaatggttatgtaaacaggtctctgccaggtctgattggatgccacaggaaatcagtctattggcatgtgattggaatgggcaccactcctgaagtgcactcaatattcctcgaaggtcacacatttcttgtgaggaaccatcgccaggcgtccttggaaatctcgccaataactttccttactgctcaaacactcttgatggaccttggacagtttctactgttttgtcatatctcttcccaccaacatgatggcatggaagcttatgtcaaagtagacagctgtccagaggaaccccaactacgaatgaaaaataatgaagaagcggaagactatgatgatgatcttactgattctgaaatggatgtggtcaggtttgatgatgacaactctccttcctttatccaaattcgctcagttgccaagaagcatcctaaaacttgggtacattacattgctgctgaagaggaggactgggactatgctcccttagtcctcgcccccgatgacagaagttataaaagtcaatatttgaacaatggccctcagcggattggtaggaagtacaaaaaagtccgatttatggcatacacagatgaaacctttaagactcgtgaagctattcagcatgaatcaggaatcttgggacctttactttatggggaagttggagacacactgttgattatatttaagaatcaagcaagcagaccatataacatctaccctcacggaatcactgatgtccgtcctttgtattcaaggagattaccaaaaggtgtaaaacatttgaaggattttccaattctgccaggagaaatattcaaatataaatggacagtgactgtagaagatgggccaactaaatcagatcctcggtgcctgacccgctattactctagtttcgttaatatggagagagatctagcttcaggactcattggccctctcctcatctgctacaaagaatctgtagatcaaagaggaaaccagataatgtcagacaagaggaatgtcatcctgttttctgtatttgatgagaaccgaagctggtacctcacagagaatatacaacgctttctccccaatccagctggagtgcagcttgaggatccagagttccaagcctccaacatcatgcacagcatcaatggctatgtttttgatagtttgcagttgtcagtttgtttgcatgaggtggcatactggtacattctaagcattggagcacagactgacttcctttctgtcttcttctctggatataccttcaaacacaaaatggtctatgaagacacactcaccctattcccattctcaggagaaactgtcttcatgtcgatggaaaacccaggtctatggattctggggtgccacaactcagactttcggaacagaggcatgaccgccttactgaaggtttctagttgtgacaagaacactggtgattattacgaggacagttatgaagatatttcagcatacttgctgagtaaaaacaatgccattgaaccaagaagcttctcccagaatcgccatcaacgggaaataactcgtactactcttcagtcagatcaagaggaaattgactatgatgataccatatcagttgaaatgaagaaggaagattttgacatttatgatgaggatgaaaatcagagcccccgcagctttcaaaagaaaacacgacactattttattgctgcagtggagaggctctgggattatgggatgagtagctccccacatgttctaagaaacagggctcagagtggcagtgtccctcagttcaagaaagttgttttccaggaatttactgatggctcctttactcagcccttataccgtggagaactaaatgaacatttgggactcctggggccatatataagagcagaagttgaagataatatcatggtaactttcagaaatcaggcctctcgtccctattccttctattctagccttatttcttatgaggaagatcagaggcaaggagcagaacctagaaaaaactttgtcaagcctaatgaaaccaaaacttacttttggaaagtgcaacatcatatggcacccactaaagatgagtttgactgcaaagcctgggcttatttctctgatgttgacctggaaaaagatgtgcactcaggcctgattggaccccttctggtctgccacactaacacactgaaccctgctcatgggagacaagtgacagtacaggaatttgctctgtttttcaccatctttgatgagaccaaaagctggtacttcactgaaaatatggaaagaaactgcagggctccctgcaatatccagatggaagatcccacttttaaagagaattatcgcttccatgcaatcaatggctacataatggatacactacctggcttagtaatggctcaggatcaaaggattcgatggtatctgctcagcatgggcagcaatgaaaacatccattctattcatttcagtggacatgtgttcactgtacgaaaaaaagaggagtataaaatggcactgtacaatctctatccaggtgtttttgagacagtggaaatgttaccatccaaagctggaatttggcgggtggaatgccttattggcgagcatctacatgctgggatgagcacactttttctggtgtacagcaataagtgtcagactcccctgggaatggcttctggacacattagagattttcagattacagcttcaggacaatatggacagtgggccccaaagctggccagacttcattattccggatcaatcaatgcctggagcaccaaggagcccttttcttggatcaaggtggatctgttggcaccaatgattattcacggcatcaagacccagggtgcccgtcagaagttctccagcctctacatctctcagtttatcatcatgtatagtcttgatgggaagaagtggcagacttatcgaggaaattccactggaaccttaatggtcttctttggcaatgtggattcatctgggataaaacacaatatttttaaccctccaattattgctcgatacatccgtttgcacccaactcattatagcattcgcagcactcttcgcatggagttgatgggctgtgatttaaatagttgcagcatgccattgggaatggagagtaaagcaatatcagatgcacagattactgcttcatcctactttaccaatatgtttgccacctggtctccttcaaaagctcgacttcacctccaagggaggagtaatgcctggagacctcaggtgaataatccaaaagagtggctgcaagtggacttccagaagacaatgaaagtcacaggagtaactactcagggagtaaaatctctgcttaccagcatgtatgtgaaggagttcctcatctccagcagtcaagatggccatcagtggactctcttttttcagaatggcaaagtaaaggtttttcagggaaatcaagactccttcacacctgtggtgaactctctagacccaccgttactgactcgctaccttcgaattcacccccagagttgggtgcaccagattgccctgaggatggaggttctgggctgcgaggcacaggacctctactag

SEQ ID NO: 7 - protein, 1452 aa, synthetic construct
  REGION 1..1452: note = Amino acid sequences of FVIII variants
MQIELSTCFFLCLLRFCFSATRRYYLGAVELSWDYMQSDLGELPVDARFPPRVPKSFPFNTSVVYKKTLFVEFTDHLFNIAKPRPPWMGLLGPTIQAEVYDTVVITLKNMASHPVSLHAVGVSYWKASEGAEYDDQTSQREKEDDKVFPGGSHTYVWQVLKENGPMASDPLCLTYSYLSHVDLVKDLNSGLIGALLVCREGSLAKEKTQTLHKFILLFAVFDEGKSWHSETKNSLMQDRDAASARAWPKMHTVNGYVNRSLPGLIGCHRKSVYWHVIGMGTTPEVHSIFLEGHTFLVRNHRQASLEISPITFLTAQTLLMDLGQFLLFCHISSHQHDGMEAYVKVDSCPEEPQLRMKNNEEAEDYDDDLTDSEMDVVRFDDDNSPSFIQIRSVAKKHPKTWVHYIAAEEEDWDYAPLVLAPDDRSYKSQYLNNGPQRIGRKYKKVRFMAYTDETFKTREAIQHESGILGPLLYGEVGDTLLIIFKNQASRPYNIYPHGITDVRPLYSRRLPKGVKHLKDFPILPGEIFKYKWTVTVEDGPTKSDPRCLTRYYSSFVNMERDLASGLIGPLLICYKESVDQRGNQIMSDKRNVILFSVFDENRSWYLTENIQRFLPNPAGVQLEDPEFQASNIMHSINGYVFDSLQLSVCLHEVAYWYILSIGAQTDFLSVFFSGYTFKHKMVYEDTLTLFPFSGETVFMSMENPGLWILGCHNSDFRNRGMTALLKVSSCDKNTGDYYEDSYEDISAYLLSKNNAIEPRSFSQNRHQREITRTTLQSDQEEIDYDDTISVEMKKEDFDIYDEDENQSPRSFQKKTRHYFIAAVERLWDYGMSSSPHVLRNRAQSGSVPQFKKVVFQEFTDGSFTQPLYRGELNEHLGLLGPYIRAEVEDNIMVTFRNQASRPYSFYSSLISYEEDQRQGAEPRKNFVKPNETKTYFWKVQHHMAPTKDEFDCKAWAYFSDVDLEKDVHSGLIGPLLVCHTNTLNPAHGRQVTVQEFALFFTIFDETKSWYFTENMERNCRAPCNIQMEDPTFKENYRFHAINGYIMDTLPGLVMAQDQRIRWYLLSMGSNENIHSIHFSGHVFTVRKKEEYKMALYNLYPGVFETVEMLPSKAGIWRVECLIGEHLHAGMSTLFLVYSNKCQTPLGMASGHIRDFQITASGQYGQWAPKLARLHYSGSINAWSTKEPFSWIKVDLLAPMIIHGIKTQGARQKFSSLYISQFIIMYSLDGKKWQTYRGNSTGTLMVFFGNVDSSGIKHNIFNPPIIARYIRLHPTHYSIRSTLRMELMGCDLNSCSMPLGMESKAISDAQITASSYFTNMFATWSPSKARLHLQGRSNAWRPQVNNPKEWLQVDFQKTMKVTGVTTQGVKSLLTSMYVKEFLISSSQDGHQWTLFFQNGKVKVFQGNQDSFTPVVNSLDPPLLTRYLRIHPQSWVHQIALRMEVLGCEAQDLY

SEQ ID NO: 8 - DNA, 61 bp, synthetic construct
  misc_feature 1..61: note = Poly A
  source 1..61: mol_type = other DNA
tcgcgaataaaagatctttattttcattagatctgtgtgttggttttttgtgtgatgcagc

SEQ ID NO: 9 - DNA, 4793 bp, synthetic construct
  misc_feature 1..4793: note = Isolated nucleic acid molecules, i.e. sequences between ITRs: sequence ofpromoter-kozac-codon optimized FVIII nucleic acid- k13 poly A
  source 1..4793: mol_type = other DNA
gctaaaatgggcaaacatgctgtttactgagctgggcacaatgacctttggcgagctggacagagggccgggtgctgacgtgcaggcgggtgggctgacctttaaacttgtttgctcctccgataaccggggtgaccttggttaatcattaaccagcaatggggttaataattttccagatctctctgagcaatagtataaaacaagaggtatcactcatttcagatcaggcttctcagaggtccccacccaatacatctccagtcatgcagattgagctgagcacctgcttcttcctgtgcctgctgaggttctgcttctctgccaccaggagatactacctgggggctgtggagctgagctgggactacatgcagtctgacctgggggagctgcctgtggatgccaggttcccccccagagtgcccaagagcttccccttcaacacctctgtggtgtacaagaagaccctgtttgtggagttcactgaccacctgttcaacattgccaagcccaggcccccctggatgggcctgctgggccccaccatccaggctgaggtgtatgacactgtggtgatcaccctgaagaacatggccagccaccctgtgagcctgcatgctgtgggggtgagctactggaaggcctctgagggggctgagtatgatgaccagaccagccagagggagaaggaggatgacaaggtgttccctgggggcagccacacctatgtgtggcaggtgctgaaggagaatggccccatggcctctgaccccctgtgcctgacctacagctacctgagccatgtggacctggtgaaggacctgaactctggcctgattggggccctgctggtgtgcagggagggcagcctggccaaggagaagacccagaccctgcacaagttcatcctgctgtttgctgtgtttgatgagggcaagagctggcactctgaaaccaagaacagcctgatgcaggacagggatgctgcctctgccagggcctggcccaagatgcacactgtgaatggctatgtgaacaggagcctgcctggcctgattggctgccacaggaagtctgtgtactggcatgtgattggcatgggcaccacccctgaggtgcacagcatcttcctggagggccacaccttcctggtcaggaaccacaggcaggccagcctggagatcagccccatcaccttcctgactgcccagaccctgctgatggacctgggccagttcctgctgttctgccacatcagcagccaccagcatgatggcatggaggcctatgtgaaggtggacagctgccctgaggagccccagctgaggatgaagaacaatgaggaggctgaggactatgatgatgacctgactgactctgagatggatgtggtgaggtttgatgatgacaacagccccagcttcatccagatcaggtctgtggccaagaagcaccccaagacctgggtgcactacattgctgctgaggaggaggactgggactatgcccccctggtgctggcccctgatgacaggagctacaagagccagtacctgaacaatggcccccagaggattggcaggaagtacaagaaggtcaggttcatggcctacactgatgaaaccttcaagaccagggaggccatccagcatgagtctggcatcctgggccccctgctgtatggggaggtgggggacaccctgctgatcatcttcaagaaccaggccagcaggccctacaacatctacccacatggcatcactgatgtgaggcccctgtacagcaggaggctgcccaagggggtgaagcacctgaaggacttccccatcctgcctggggagatcttcaagtacaagtggactgtgactgtggaggatggccccaccaagtctgaccccaggtgcctgaccagatactacagcagctttgtgaacatggagagggacctggcctctggcctgattggccccctgctgatctgctacaaggagtctgtggaccagaggggcaaccagatcatgtctgacaagaggaatgtgatcctgttctctgtgtttgatgagaacaggagctggtacctgactgagaacatccagaggttcctgcccaaccctgctggggtgcagctggaggaccctgagttccaggccagcaacatcatgcacagcatcaatggctatgtgtttgacagcctgcagctgtctgtgtgcctgcatgaggtggcctactggtacatcctgagcattggggcccagactgacttcctgtctgtgttcttctctggctacaccttcaagcacaagatggtgtatgaggacaccctgaccctgttccccttctctggggagactgtgttcatgagcatggagaaccctggcctgtggattctgggctgccacaactctgacttcaggaacaggggcatgactgccctgctgaaagtctccagctgtgacaagaacactggggactactatgaggacagctatgaggacatctctgcctacctgctgagcaagaacaatgccattgagcccaggagcttcagccagaatgccactaatgtgtctaacaacagcaacaccagcaatgacagcaatgtgtctcccccagtgctgaagaggcaccagagggagatcaccaggaccaccctgcagtctgaccaggaggagattgactatgatgacaccatctctgtggagatgaagaaggaggactttgacatctacgacgaggacgagaaccagagccccaggagcttccagaagaagaccaggcactacttcattgctgctgtggagaggctgtgggactatggcatgagcagcagcccccatgtgctgaggaacagggcccagtctggctctgtgccccagttcaagaaggtggtgttccaggagttcactgatggcagcttcacccagcccctgtacagaggggagctgaatgagcacctgggcctgctgggcccctacatcagggctgaggtggaggacaacatcatggtgaccttcaggaaccaggccagcaggccctacagcttctacagcagcctgatcagctatgaggaggaccagaggcagggggctgagcccaggaagaactttgtgaagcccaatgaaaccaagacctacttctggaaggtgcagcaccacatggcccccaccaaggatgagtttgactgcaaggcctgggcctacttctctgatgtggacctggagaaggatgtgcactctggcctgattggccccctgctggtgtgccacaccaacaccctgaaccctgcccatggcaggcaggtgactgtgcaggagtttgccctgttcttcaccatctttgatgaaaccaagagctggtacttcactgagaacatggagaggaactgcagggccccctgcaacatccagatggaggaccccaccttcaaggagaactacaggttccatgccatcaatggctacatcatggacaccctgcctggcctggtgatggcccaggaccagaggatcaggtggtacctgctgagcatgggcagcaatgagaacatccacagcatccacttctctggccatgtgttcactgtgaggaagaaggaggagtacaagatggccctgtacaacctgtaccctggggtgtttgagactgtggagatgctgcccagcaaggctggcatctggagggtggagtgcctgattggggagcacctgcatgctggcatgagcaccctgttcctggtgtacagcaacaagtgccagacccccctgggcatggcctctggccacatcagggacttccagatcactgcctctggccagtatggccagtgggcccccaagctggccaggctgcactactctggcagcatcaatgcctggagcaccaaggagcccttcagctggatcaaggtggacctgctggcccccatgatcatccatggcatcaagacccagggggccaggcagaagttcagcagcctgtacatcagccagttcatcatcatgtacagcctggatggcaagaagtggcagacctacaggggcaacagcactggcacactgatggtgttctttggcaatgtggacagctctggcatcaagcacaacatcttcaacccccccatcattgccagatacatcaggctgcaccccacccactacagcatcaggagcaccctgaggatggagctgatgggctgtgacctgaacagctgcagcatgcccctgggcatggagagcaaggccatctctgatgcccagatcactgccagcagctacttcaccaacatgtttgccacctggagccccagcaaggccaggctgcacctgcagggcaggagcaatgcctggaggccccaggtcaacaaccccaaggagtggctgcaggtggacttccagaagaccatgaaggtgactggggtgaccacccagggggtgaagagcctgctgaccagcatgtatgtgaaggagttcctgatcagcagcagccaggatggccaccagtggaccctgttcttccagaatggcaaggtgaaggtgttccagggcaaccaggacagcttcacccctgtggtgaacagcctggacccccccctgctgaccagatacctgaggattcacccccagagctgggtgcaccagattgccctgaggatggaggtgctgggctgtgaggcccaggacctgtactgagaatgcataaattgtaaatttattgacaaacaataaacaacaataaacaactgaaatgagtggctatgtattaaagaggggctggggggttgggttggccgc

SEQ ID NO: 10 - DNA, 255 bp, synthetic construct
  misc_feature 1..255: note = Promoter
  source 1..255: mol_type = other DNA
aatgactcctttcggtaagtgcagtggaagctgtacactgcccaggcaaagcgtccgggcagcgtaggcgggcgactcagatcccagccagtggacttagcccctgtttgctcctccgataactggggtgaccttggttaatattcaccagcagcctcccccgttgcccctctggatccactgcttaaatacggacgaggacagggccctgtctcctcagcttcaggcaccaccactgacctgggacagtgaatc